European Patent Specification EP 4 023 232 B1, published September 17, 2025. Title: PHARMACEUTICAL COMPOSITION FOR TREATING CANCER COMPRISING ONCOLYTIC VIRUS, IMMUNE CHECKPOINT INHIBITOR AND HYDROXYUREA. Applicant: Bionoxx Inc. Pusan National University Industry-University Cooperation Foundation. The sequence listing filed with the application follows.

SEQUENCE LISTING (1 sequence)

SEQ ID NO: 1 - DNA, 1131 bp, Artificial Sequence
  nucleotide sequence for mutated HSV-TK of WOTS-418
atggcttcgtacccctgccatcaacacgcgtctgcgttcgaccaggctgcgcgttctcgcggccatagcaaccgacgtacggcgttgcgccctcgccggcagcaagaagccacggaagtccgcctggagcagaaaatgcccacgctactgcgggtttatatagacggtcctcacgggatggggaaaaccaccaccacgcaactgctggtggccctgggttcgcgcgacgatatcgtctacgtacccgagccgatgacttactggcaggtgctgggggcttccgagacaatcgcgaacatctacaccacacaacaccgcctcgaccagggtgagatatcggccggggacgcggcggtggtaatgacaagcgcccagataacaatgggcatgccttatgccgtgaccgacgccgttctggctcctcatgtcggtggtgaggctgggagttcacatgccccgcccccggccctcaccctcatcttcgaccgccatcccatctacgccctcctgtgctacccggccgcgcgataccttatgggcagcatgacccctcaggccgtgctggcgttcgtggccctcatcccgccgaccttgcccggcacaaacatcgtgttgggggcccttccggaggacagacacatcgaccgcctggccaaacgccagcgccccggcgagcggcttgacctggctatgctggccgcgattcgccgcgtttacgggctgcttgccaatacggtgcggtatctgcagggcggcgggtcgtggtgggaggattggggacagctttcggggacggccgtgccgccccagggtgccgagccccagagcaacgcgggcccacgaccccatatcggggacacgttatttaccctgtttcgggcccccgagttgctggcccccaacggcgacctgtataacgtgtttgcctgggccttggacgtcttggccaaacgcctccgtcccatgcacgtctttatcctggattacgaccaatcgcccgccggctgccgggacgccctgctgcaacttacctccgggatggtccagacccacgtcaccaccccaggctccataccgacgatctgcgacctggcgcgcacgtttgcccgggagatgggggaggctaactaa